European Patent Application EP 4 165 999 A1, published April 19, 2023. Title: A method for preparing a dairy product having a stable content of galacto-oligosaccharide(s). Applicant: DuPont Nutrition Biosciences ApS. The sequence listing filed with the application follows.

SEQUENCE LISTING (23 sequences)

SEQ ID NO: 1 - protein, 887 aa, Bifidobacterium bifidum
VEDATRSDSTTQMSSTPEVVYSSAVDSKQNRTSDFDANWKFMLSDSVQAQDPAFDDSAWQQVDLPHDYSITQKYSQSNEAESAYLPGGTGWYRKSFTIDRDLAGKRIAINFDGVYMNATVWFNGVKLGTHPYGYSPFSFDLTGNAKFGGENTIVVKVENRLPSSRWYSGSGIYRDVTLTVTDGVHVGNNGVAIKTPSLATQNGGDVTMNLTTKVANDTEAAANITLKQTVFPKGGKTDAAIGTVTTASKSIAAGASADVTSTITAASPKLWSIKNPNLYTVRTEVLNGGKVLDTYDTEYGFRWTGFDATSGFSLNGEKVKLKGVSMHHDQGSLGAVANRRAIERQVEILQKMGVNSIRTTHNPAAKALIDVCNEKGVLVVEEVFDMWNRSKNGNTEDYGKWFGQAIAGDNAVLGGDKDETWAKFDLTSTINRDRNAPSVIMWSLGNEMMEGISGSVSGFPATSAKLVAWTKAADSTRPMTYGDNKIKANWNESNTMGDNLTANGGVVGTNYSDGANYDKIRTTHPSWAIYGSETASAINSRGIYNRTTGGAQSSDKQLTSYDNSAVGWGAVASSAWYDVVQRDFVAGTYVWTGFDYLGEPTPWNGTGSGAVGSWPSPKNSYFGIVDTAGFPKDTYYFYQSQWNDDVHTLHILPAWNENVVAKGSGNNVPVVVYTDAAKVKLYFTPKGSTEKRLIGEKSFTKKTTAAGYTYQVYEGSDKDSTAHKNMYLTWNVPWAEGTISAEAYDENNRLIPEGSTEGNASVTTTGKAAKLKADADRKTITADGKDLSYIEVDVTDANGHIVPDAANRVTFDVKGAGKLVGVDNGSSPDHDSYQADNRKAFSGKVLAIVQSTKEAGEITVTAKADGLQSSTVKIATTAVPGTSTEKT

SEQ ID NO: 2 - protein, 965 aa, Bifidobacterium bifidum
VEDATRSDSTTQMSSTPEVVYSSAVDSKQNRTSDFDANWKFMLSDSVQAQDPAFDDSAWQQVDLPHDYSITQKYSQSNEAESAYLPGGTGWYRKSFTIDRDLAGKRIAINFDGVYMNATVWFNGVKLGTHPYGYSPFSFDLTGNAKFGGENTIVVKVENRLPSSRWYSGSGIYRDVTLTVTDGVHVGNNGVAIKTPSLATQNGGDVTMNLTTKVANDTEAAANITLKQTVFPKGGKTDAAIGTVTTASKSIAAGASADVTSTITAASPKLWSIKNPNLYTVRTEVLNGGKVLDTYDTEYGFRWTGFDATSGFSLNGEKVKLKGVSMHHDQGSLGAVANRRAIERQVEILQKMGVNSIRTTHNPAAKALIDVCNEKGVLVVEEVFDMWNRSKNGNTEDYGKWFGQAIAGDNAVLGGDKDETWAKFDLTSTINRDRNAPSVIMWSLGNEMMEGISGSVSGFPATSAKLVAWTKAADSTRPMTYGDNKIKANWNESNTMGDNLTANGGVVGTNYSDGANYDKIRTTHPSWAIYGSETASAINSRGIYNRTTGGAQSSDKQLTSYDNSAVGWGAVASSAWYDVVQRDFVAGTYVWTGFDYLGEPTPWNGTGSGAVGSWPSPKNSYFGIVDTAGFPKDTYYFYQSQWNDDVHTLHILPAWNENVVAKGSGNNVPVVVYTDAAKVKLYFTPKGSTEKRLIGEKSFTKKTTAAGYTYQVYEGSDKDSTAHKNMYLTWNVPWAEGTISAEAYDENNRLIPEGSTEGNASVTTTGKAAKLKADADRKTITADGKDLSYIEVDVTDANGHIVPDAANRVTFDVKGAGKLVGVDNGSSPDHDSYQADNRKAFSGKVLAIVQSTKEAGEITVTAKADGLQSSTVKIATTAVPGTSTEKTVRSFYYSRNYYVKTGNKPILPSDVEVRYSDGTSDRQNVTWDAVSDDQIAKAGSFSVAGTVAGQKISVRVTMIDEIGAL

SEQ ID NO: 3 - protein, 1038 aa, Bifidobacterium bifidum
VEDATRSDSTTQMSSTPEVVYSSAVDSKQNRTSDFDANWKFMLSDSVQAQDPAFDDSAWQQVDLPHDYSITQKYSQSNEAESAYLPGGTGWYRKSFTIDRDLAGKRIAINFDGVYMNATVWFNGVKLGTHPYGYSPFSFDLTGNAKFGGENTIVVKVENRLPSSRWYSGSGIYRDVTLTVTDGVHVGNNGVAIKTPSLATQNGGDVTMNLTTKVANDTEAAANITLKQTVFPKGGKTDAAIGTVTTASKSIAAGASADVTSTITAASPKLWSIKNPNLYTVRTEVLNGGKVLDTYDTEYGFRWTGFDATSGFSLNGEKVKLKGVSMHHDQGSLGAVANRRAIERQVEILQKMGVNSIRTTHNPAAKALIDVCNEKGVLVVEEVFDMWNRSKNGNTEDYGKWFGQAIAGDNAVLGGDKDETWAKFDLTSTINRDRNAPSVIMWSLGNEMMEGISGSVSGFPATSAKLVAWTKAADSTRPMTYGDNKIKANWNESNTMGDNLTANGGVVGTNYSDGANYDKIRTTHPSWAIYGSETASAINSRGIYNRTTGGAQSSDKQLTSYDNSAVGWGAVASSAWYDVVQRDFVAGTYVWTGFDYLGEPTPWNGTGSGAVGSWPSPKNSYFGIVDTAGFPKDTYYFYQSQWNDDVHTLHILPAWNENVVAKGSGNNVPVVVYTDAAKVKLYFTPKGSTEKRLIGEKSFTKKTTAAGYTYQVYEGSDKDSTAHKNMYLTWNVPWAEGTISAEAYDENNRLIPEGSTEGNASVTTTGKAAKLKADADRKTITADGKDLSYIEVDVTDANGHIVPDAANRVTFDVKGAGKLVGVDNGSSPDHDSYQADNRKAFSGKVLAIVQSTKEAGEITVTAKADGLQSSTVKIATTAVPGTSTEKTVRSFYYSRNYYVKTGNKPILPSDVEVRYSDGTSDRQNVTWDAVSDDQIAKAGSFSVAGTVAGQKISVRVTMIDEIGALLNYSASTPVGTPAVLPGSRPAVLPDGTVTSANFAVHWTKPADTVYNTAGTVKVPGTATVFGKEFKVTATIRVQ

SEQ ID NO: 4 - protein, 1142 aa, Bifidobacterium bifidum
VEDATRSDSTTQMSSTPEVVYSSAVDSKQNRTSDFDANWKFMLSDSVQAQDPAFDDSAWQQVDLPHDYSITQKYSQSNEAESAYLPGGTGWYRKSFTIDRDLAGKRIAINFDGVYMNATVWFNGVKLGTHPYGYSPFSFDLTGNAKFGGENTIVVKVENRLPSSRWYSGSGIYRDVTLTVTDGVHVGNNGVAIKTPSLATQNGGDVTMNLTTKVANDTEAAANITLKQTVFPKGGKTDAAIGTVTTASKSIAAGASADVTSTITAASPKLWSIKNPNLYTVRTEVLNGGKVLDTYDTEYGFRWTGFDATSGFSLNGEKVKLKGVSMHHDQGSLGAVANRRAIERQVEILQKMGVNSIRTTHNPAAKALIDVCNEKGVLVVEEVFDMWNRSKNGNTEDYGKWFGQAIAGDNAVLGGDKDETWAKFDLTSTINRDRNAPSVIMWSLGNEMMEGISGSVSGFPATSAKLVAWTKAADSTRPMTYGDNKIKANWNESNTMGDNLTANGGVVGTNYSDGANYDKIRTTHPSWAIYGSETASAINSRGIYNRTTGGAQSSDKQLTSYDNSAVGWGAVASSAWYDVVQRDFVAGTYVWTGFDYLGEPTPWNGTGSGAVGSWPSPKNSYFGIVDTAGFPKDTYYFYQSQWNDDVHTLHILPAWNENVVAKGSGNNVPVVVYTDAAKVKLYFTPKGSTEKRLIGEKSFTKKTTAAGYTYQVYEGSDKDSTAHKNMYLTWNVPWAEGTISAEAYDENNRLIPEGSTEGNASVTTTGKAAKLKADADRKTITADGKDLSYIEVDVTDANGHIVPDAANRVTFDVKGAGKLVGVDNGSSPDHDSYQADNRKAFSGKVLAIVQSTKEAGEITVTAKADGLQSSTVKIATTAVPGTSTEKTVRSFYYSRNYYVKTGNKPILPSDVEVRYSDGTSDRQNVTWDAVSDDQIAKAGSFSVAGTVAGQKISVRVTMIDEIGALLNYSASTPVGTPAVLPGSRPAVLPDGTVTSANFAVHWTKPADTVYNTAGTVKVPGTATVFGKEFKVTATIRVQRSQVTIGSSVSGNALRLTQNIPADKQSDTLDAIKDGSTTVDANTGGGANPSAWTNWAYSKAGHNTAEITFEYATEQQLGQIVMYFFRDSNAVRFPDAGKTKIQI

SEQ ID NO: 5 - protein, 1211 aa, Bifidobacterium bifidum
VEDATRSDSTTQMSSTPEVVYSSAVDSKQNRTSDFDANWKFMLSDSVQAQDPAFDDSAWQQVDLPHDYSITQKYSQSNEAESAYLPGGTGWYRKSFTIDRDLAGKRIAINFDGVYMNATVWFNGVKLGTHPYGYSPFSFDLTGNAKFGGENTIVVKVENRLPSSRWYSGSGIYRDVTLTVTDGVHVGNNGVAIKTPSLATQNGGDVTMNLTTKVANDTEAAANITLKQTVFPKGGKTDAAIGTVTTASKSIAAGASADVTSTITAASPKLWSIKNPNLYTVRTEVLNGGKVLDTYDTEYGFRWTGFDATSGFSLNGEKVKLKGVSMHHDQGSLGAVANRRAIERQVEILQKMGVNSIRTTHNPAAKALIDVCNEKGVLVVEEVFDMWNRSKNGNTEDYGKWFGQAIAGDNAVLGGDKDETWAKFDLTSTINRDRNAPSVIMWSLGNEMMEGISGSVSGFPATSAKLVAWTKAADSTRPMTYGDNKIKANWNESNTMGDNLTANGGVVGTNYSDGANYDKIRTTHPSWAIYGSETASAINSRGIYNRTTGGAQSSDKQLTSYDNSAVGWGAVASSAWYDVVQRDFVAGTYVWTGFDYLGEPTPWNGTGSGAVGSWPSPKNSYFGIVDTAGFPKDTYYFYQSQWNDDVHTLHILPAWNENVVAKGSGNNVPVVVYTDAAKVKLYFTPKGSTEKRLIGEKSFTKKTTAAGYTYQVYEGSDKDSTAHKNMYLTWNVPWAEGTISAEAYDENNRLIPEGSTEGNASVTTTGKAAKLKADADRKTITADGKDLSYIEVDVTDANGHIVPDAANRVTFDVKGAGKLVGVDNGSSPDHDSYQADNRKAFSGKVLAIVQSTKEAGEITVTAKADGLQSSTVKIATTAVPGTSTEKTVRSFYYSRNYYVKTGNKPILPSDVEVRYSDGTSDRQNVTWDAVSDDQIAKAGSFSVAGTVAGQKISVRVTMIDEIGALLNYSASTPVGTPAVLPGSRPAVLPDGTVTSANFAVHWTKPADTVYNTAGTVKVPGTATVFGKEFKVTATIRVQRSQVTIGSSVSGNALRLTQNIPADKQSDTLDAIKDGSTTVDANTGGGANPSAWTNWAYSKAGHNTAEITFEYATEQQLGQIVMYFFRDSNAVRFPDAGKTKIQISADGKNWTDLAATETIAAQESSDRVKPYTYDFAPVGATFVKVTVTNADTTTPSGVVCAGLTEIELKTAT

SEQ ID NO: 6 - protein, 1296 aa, Bifidobacterium bifidum
VEDATRSDSTTQMSSTPEVVYSSAVDSKQNRTSDFDANWKFMLSDSVQAQDPAFDDSAWQQVDLPHDYSITQKYSQSNEAESAYLPGGTGWYRKSFTIDRDLAGKRIAINFDGVYMNATVWFNGVKLGTHPYGYSPFSFDLTGNAKFGGENTIVVKVENRLPSSRWYSGSGIYRDVTLTVTDGVHVGNNGVAIKTPSLATQNGGDVTMNLTTKVANDTEAAANITLKQTVFPKGGKTDAAIGTVTTASKSIAAGASADVTSTITAASPKLWSIKNPNLYTVRTEVLNGGKVLDTYDTEYGFRWTGFDATSGFSLNGEKVKLKGVSMHHDQGSLGAVANRRAIERQVEILQKMGVNSIRTTHNPAAKALIDVCNEKGVLVVEEVFDMWNRSKNGNTEDYGKWFGQAIAGDNAVLGGDKDETWAKFDLTSTINRDRNAPSVIMWSLGNEMMEGISGSVSGFPATSAKLVAWTKAADSTRPMTYGDNKIKANWNESNTMGDNLTANGGVVGTNYSDGANYDKIRTTHPSWAIYGSETASAINSRGIYNRTTGGAQSSDKQLTSYDNSAVGWGAVASSAWYDVVQRDFVAGTYVWTGFDYLGEPTPWNGTGSGAVGSWPSPKNSYFGIVDTAGFPKDTYYFYQSQWNDDVHTLHILPAWNENVVAKGSGNNVPVVVYTDAAKVKLYFTPKGSTEKRLIGEKSFTKKTTAAGYTYQVYEGSDKDSTAHKNMYLTWNVPWAEGTISAEAYDENNRLIPEGSTEGNASVTTTGKAAKLKADADRKTITADGKDLSYIEVDVTDANGHIVPDAANRVTFDVKGAGKLVGVDNGSSPDHDSYQADNRKAFSGKVLAIVQSTKEAGEITVTAKADGLQSSTVKIATTAVPGTSTEKTVRSFYYSRNYYVKTGNKPILPSDVEVRYSDGTSDRQNVTWDAVSDDQIAKAGSFSVAGTVAGQKISVRVTMIDEIGALLNYSASTPVGTPAVLPGSRPAVLPDGTVTSANFAVHWTKPADTVYNTAGTVKVPGTATVFGKEFKVTATIRVQRSQVTIGSSVSGNALRLTQNIPADKQSDTLDAIKDGSTTVDANTGGGANPSAWTNWAYSKAGHNTAEITFEYATEQQLGQIVMYFFRDSNAVRFPDAGKTKIQISADGKNWTDLAATETIAAQESSDRVKPYTYDFAPVGATFVKVTVTNADTTTPSGVVCAGLTEIELKTATSKFVTNTSAALSSLTVNGTKVSDSVLAAGSYNTPAIIADVKAEGEGNASVTVLPAHDNVIRVITESEDHVTRKTFTINLGTEQEF

SEQ ID NO: 7 - protein, 453 aa, Bifidobacterium bifidum
  source 1..453: note = Glycoside hydrolase catalytic core
QNRTSDFDANWKFMLSDSVQAQDPAFDDSAWQQVDLPHDYSITQKYSQSNEAESAYLPGGTGWYRKSFTIDRDLAGKRIAINFDGVYMNATVWFNGVKLGTHPYGYSPFSFDLTGNAKFGGENTIVVKVENRLPSSRWYSGSGIYRDVTLTVTDGVHVGNNGVAIKTPSLATQNGGDVTMNLTTKVANDTEAAANITLKQTVFPKGGKTDAAIGTVTTASKSIAAGASADVTSTITAASPKLWSIKNPNLYTVRTEVLNGGKVLDTYDTEYGFRWTGFDATSGFSLNGEKVKLKGVSMHHDQGSLGAVANRRAIERQVEILQKMGVNSIRTTHNPAAKALIDVCNEKGVLVVEEVFDMWNRSKNGNTEDYGKWFGQAIAGDNAVLGGDKDETWAKFDLTSTINRDRNAPSVIMWSLGNEMMEGISGSVSGFPATSAKLVAWTKAADSTRPMTY

SEQ ID NO: 8 - DNA, 5160 bp, Bifidobacterium bifidum
  source 1..5160: mol_type = other DNA
gcagttgaagatgcaacaagaagcgatagcacaacacaaatgtcatcaacaccggaagttgtttattcatcagcggtcgatagcaaacaaaatcgcacaagcgattttgatgcgaactggaaatttatgctgtcagatagcgttcaagcacaagatccggcatttgatgattcagcatggcaacaagttgatctgccgcatgattatagcatcacacagaaatatagccaaagcaatgaagcagaatcagcatatcttccgggaggcacaggctggtatagaaaaagctttacaattgatagagatctggcaggcaaacgcattgcgattaattttgatggcgtctatatgaatgcaacagtctggtttaatggcgttaaactgggcacacatccgtatggctattcaccgttttcatttgatctgacaggcaatgcaaaatttggcggagaaaacacaattgtcgtcaaagttgaaaatagactgccgtcatcaagatggtattcaggcagcggcatttatagagatgttacactgacagttacagatggcgttcatgttggcaataatggcgtcgcaattaaaacaccgtcactggcaacacaaaatggcggagatgtcacaatgaacctgacaacaaaagtcgcgaatgatacagaagcagcagcgaacattacactgaaacagacagtttttccgaaaggcggaaaaacggatgcagcaattggcacagttacaacagcatcaaaatcaattgcagcaggcgcatcagcagatgttacaagcacaattacagcagcaagcccgaaactgtggtcaattaaaaacccgaacctgtatacagttagaacagaagttctgaacggaggcaaagttctggatacatatgatacagaatatggctttcgctggacaggctttgatgcaacatcaggcttttcactgaatggcgaaaaagtcaaactgaaaggcgttagcatgcatcatgatcaaggctcacttggcgcagttgcaaatagacgcgcaattgaaagacaagtcgaaatcctgcaaaaaatgggcgtcaatagcattcgcacaacacataatccggcagcaaaagcactgattgatgtctgcaatgaaaaaggcgttctggttgtcgaagaagtctttgatatgtggaaccgcagcaaaaatggcaacacggaagattatggcaaatggtttggccaagcaattgcaggcgataatgcagttctgggaggcgataaagatgaaacatgggcgaaatttgatcttacatcaacaattaaccgcgatagaaatgcaccgtcagttattatgtggtcactgggcaatgaaatgatggaaggcatttcaggctcagtttcaggctttccggcaacatcagcaaaactggttgcatggacaaaagcagcagattcaacaagaccgatgacatatggcgataacaaaattaaagcgaactggaacgaatcaaatacaatgggcgataatctgacagcaaatggcggagttgttggcacaaattattcagatggcgcaaactatgataaaattcgtacaacacatccgtcatgggcaatttatggctcagaaacagcatcagcgattaatagccgtggcatttataatagaacaacaggcggagcacaatcatcagataaacagctgacaagctatgataattcagcagttggctggggagcagttgcatcatcagcatggtatgatgttgttcagagagattttgtcgcaggcacatatgtttggacaggatttgattatctgggcgaaccgacaccgtggaatggcacaggctcaggcgcagttggctcatggccgtcaccgaaaaatagctattttggcatcgttgatacagcaggctttccgaaagatacatattatttttatcagagccagtggaatgatgatgttcatacactgcatattcttccggcatggaatgaaaatgttgttgcaaaaggctcaggcaataatgttccggttgtcgtttatacagatgcagcgaaagtgaaactgtattttacaccgaaaggctcaacagaaaaaagactgatcggcgaaaaatcatttacaaaaaaaacaacagcggcaggctatacatatcaagtctatgaaggcagcgataaagattcaacagcgcataaaaacatgtatctgacatggaatgttccgtgggcagaaggcacaatttcagcggaagcgtatgatgaaaataatcgcctgattccggaaggcagcacagaaggcaacgcatcagttacaacaacaggcaaagcagcaaaactgaaagcagatgcggatcgcaaaacaattacagcggatggcaaagatctgtcatatattgaagtcgatgtcacagatgcaaatggccatattgttccggatgcagcaaatagagtcacatttgatgttaaaggcgcaggcaaactggttggcgttgataatggctcatcaccggatcatgattcatatcaagcggataaccgcaaagcattttcaggcaaagtcctggcaattgttcagtcaacaaaagaagcaggcgaaattacagttacagcaaaagcagatggcctgcaatcaagcacagttaaaattgcaacaacagcagttccgggaacaagcacagaaaaaacagtccgcagcttttattacagccgcaactattatgtcaaaacaggcaacaaaccgattctgccgtcagatgttgaagttcgctattcagatggaacaagcgatagacaaaacgttacatgggatgcagtttcagatgatcaaattgcaaaagcaggctcattttcagttgcaggcacagttgcaggccaaaaaattagcgttcgcgtcacaatgattgatgaaattggcgcactgctgaattattcagcaagcacaccggttggcacaccggcagttcttccgggatcaagaccggcagtcctgccggatggcacagtcacatcagcaaattttgcagtccattggacaaaaccggcagatacagtctataatacagcaggcacagtcaaagtaccgggaacagcaacagtttttggcaaagaatttaaagtcacagcgacaattagagttcaaagaagccaagttacaattggctcatcagtttcaggaaatgcactgagactgacacaaaatattccggcagataaacaatcagatacactggatgcgattaaagatggctcaacaacagttgatgcaaatacaggcggaggcgcaaatccgtcagcatggacaaattgggcatattcaaaagcaggccataacacagcggaaattacatttgaatatgcgacagaacaacaactgggccagatcgtcatgtatttttttcgcgatagcaatgcagttagatttccggatgctggcaaaacaaaaattcagatcagcgcagatggcaaaaattggacagatctggcagcaacagaaacaattgcagcgcaagaatcaagcgatagagtcaaaccgtatacatatgattttgcaccggttggcgcaacatttgttaaagtgacagtcacaaacgcagatacaacaacaccgtcaggcgttgtttgcgcaggcctgacagaaattgaactgaaaacagcgacaagcaaatttgtcacaaatacatcagcagcactgtcatcacttacagtcaatggcacaaaagtttcagattcagttctggcagcaggctcatataacacaccggcaattatcgcagatgttaaagcggaaggcgaaggcaatgcaagcgttacagtccttccggcacatgataatgttattcgcgtcattacagaaagcgaagatcatgtcacacgcaaaacatttacaatcaacctgggcacagaacaagaatttccggctgattcagatgaaagagattatccggcagcagatatgacagtcacagttggctcagaacaaacatcaggcacagcaacagaaggaccgaaaaaatttgcagtcgatggcaacacatcaacatattggcatagcaattggacaccgacaacagttaatgatctgtggatcgcgtttgaactgcaaaaaccgacaaaactggatgcactgagatatcttccgcgtccggcaggctcaaaaaatggcagcgtcacagaatataaagttcaggtgtcagatgatggaacaaactggacagatgcaggctcaggcacatggacaacggattatggctggaaactggcggaatttaatcaaccggtcacaacaaaacatgttagactgaaagcggttcatacatatgcagatagcggcaacgataaatttatgagcgcaagcgaaattagactgagaaaagcggtcgatacaacggatatttcaggcgcaacagttacagttccggcaaaactgacagttgatagagttgatgcagatcatccggcaacatttgcaacaaaagatgtcacagttacactgggagatgcaacactgagatatggcgttgattatctgctggattatgcaggcaatacagcagttggcaaagcaacagtgacagttagaggcattgataaatattcaggcacagtcgcgaaaacatttacaattgaactgaaaaatgcaccggcaccggaaccgacactgacatcagttagcgtcaaaacaaaaccgagcaaactgacatatgttgtcggagatgcatttgatccggcaggcctggttctgcaacatgatagacaagcagatagacctccgcaaccgctggttggcgaacaagcggatgaacgcggactgacatgcggcacaagatgcgatagagttgaacaactgcgcaaacatgaaaatagagaagcgcatagaacaggcctggatcatctggaatttgttggcgcagcagatggcgcagttggagaacaagcaacatttaaagtccatgtccatgcagatcagggagatggcagacatgatgatgcagatgaacgcgatattgatccgcatgttccggtcgatcatgcagttggcgaactggcaagagcagcatgccatcatgttattggcctgagagtcgatacacatagacttaaagcaagcggctttcaaattccggctgatgatatggcagaaatcgatcgcattacaggctttcatcgttttgaacgccatgtc

SEQ ID NO: 9 - DNA, 2661 bp, Bifidobacterium bifidum
  source 1..2661: mol_type = other DNA
gttgaagatgcaacaagaagcgatagcacaacacaaatgtcatcaacaccggaagttgtttattcatcagcggtcgatagcaaacaaaatcgcacaagcgattttgatgcgaactggaaatttatgctgtcagatagcgttcaagcacaagatccggcatttgatgattcagcatggcaacaagttgatctgccgcatgattatagcatcacacagaaatatagccaaagcaatgaagcagaatcagcatatcttccgggaggcacaggctggtatagaaaaagctttacaattgatagagatctggcaggcaaacgcattgcgattaattttgatggcgtctatatgaatgcaacagtctggtttaatggcgttaaactgggcacacatccgtatggctattcaccgttttcatttgatctgacaggcaatgcaaaatttggcggagaaaacacaattgtcgtcaaagttgaaaatagactgccgtcatcaagatggtattcaggcagcggcatttatagagatgttacactgacagttacagatggcgttcatgttggcaataatggcgtcgcaattaaaacaccgtcactggcaacacaaaatggcggagatgtcacaatgaacctgacaacaaaagtcgcgaatgatacagaagcagcagcgaacattacactgaaacagacagtttttccgaaaggcggaaaaacggatgcagcaattggcacagttacaacagcatcaaaatcaattgcagcaggcgcatcagcagatgttacaagcacaattacagcagcaagcccgaaactgtggtcaattaaaaacccgaacctgtatacagttagaacagaagttctgaacggaggcaaagttctggatacatatgatacagaatatggctttcgctggacaggctttgatgcaacatcaggcttttcactgaatggcgaaaaagtcaaactgaaaggcgttagcatgcatcatgatcaaggctcacttggcgcagttgcaaatagacgcgcaattgaaagacaagtcgaaatcctgcaaaaaatgggcgtcaatagcattcgcacaacacataatccggcagcaaaagcactgattgatgtctgcaatgaaaaaggcgttctggttgtcgaagaagtctttgatatgtggaaccgcagcaaaaatggcaacacggaagattatggcaaatggtttggccaagcaattgcaggcgataatgcagttctgggaggcgataaagatgaaacatgggcgaaatttgatcttacatcaacaattaaccgcgatagaaatgcaccgtcagttattatgtggtcactgggcaatgaaatgatggaaggcatttcaggctcagtttcaggctttccggcaacatcagcaaaactggttgcatggacaaaagcagcagattcaacaagaccgatgacatatggcgataacaaaattaaagcgaactggaacgaatcaaatacaatgggcgataatctgacagcaaatggcggagttgttggcacaaattattcagatggcgcaaactatgataaaattcgtacaacacatccgtcatgggcaatttatggctcagaaacagcatcagcgattaatagccgtggcatttataatagaacaacaggcggagcacaatcatcagataaacagctgacaagctatgataattcagcagttggctggggagcagttgcatcatcagcatggtatgatgttgttcagagagattttgtcgcaggcacatatgtttggacaggatttgattatctgggcgaaccgacaccgtggaatggcacaggctcaggcgcagttggctcatggccgtcaccgaaaaatagctattttggcatcgttgatacagcaggctttccgaaagatacatattatttttatcagagccagtggaatgatgatgttcatacactgcatattcttccggcatggaatgaaaatgttgttgcaaaaggctcaggcaataatgttccggttgtcgtttatacagatgcagcgaaagtgaaactgtattttacaccgaaaggctcaacagaaaaaagactgatcggcgaaaaatcatttacaaaaaaaacaacagcggcaggctatacatatcaagtctatgaaggcagcgataaagattcaacagcgcataaaaacatgtatctgacatggaatgttccgtgggcagaaggcacaatttcagcggaagcgtatgatgaaaataatcgcctgattccggaaggcagcacagaaggcaacgcatcagttacaacaacaggcaaagcagcaaaactgaaagcagatgcggatcgcaaaacaattacagcggatggcaaagatctgtcatatattgaagtcgatgtcacagatgcaaatggccatattgttccggatgcagcaaatagagtcacatttgatgttaaaggcgcaggcaaactggttggcgttgataatggctcatcaccggatcatgattcatatcaagcggataaccgcaaagcattttcaggcaaagtcctggcaattgttcagtcaacaaaagaagcaggcgaaattacagttacagcaaaagcagatggcctgcaatcaagcacagttaaaattgcaacaacagcagttccgggaacaagcacagaaaaaaca

SEQ ID NO: 10 - DNA, 2895 bp, Bifidobacterium bifidum
  source 1..2895: mol_type = other DNA
gttgaagatgcaacaagaagcgatagcacaacacaaatgtcatcaacaccggaagttgtttattcatcagcggtcgatagcaaacaaaatcgcacaagcgattttgatgcgaactggaaatttatgctgtcagatagcgttcaagcacaagatccggcatttgatgattcagcatggcaacaagttgatctgccgcatgattatagcatcacacagaaatatagccaaagcaatgaagcagaatcagcatatcttccgggaggcacaggctggtatagaaaaagctttacaattgatagagatctggcaggcaaacgcattgcgattaattttgatggcgtctatatgaatgcaacagtctggtttaatggcgttaaactgggcacacatccgtatggctattcaccgttttcatttgatctgacaggcaatgcaaaatttggcggagaaaacacaattgtcgtcaaagttgaaaatagactgccgtcatcaagatggtattcaggcagcggcatttatagagatgttacactgacagttacagatggcgttcatgttggcaataatggcgtcgcaattaaaacaccgtcactggcaacacaaaatggcggagatgtcacaatgaacctgacaacaaaagtcgcgaatgatacagaagcagcagcgaacattacactgaaacagacagtttttccgaaaggcggaaaaacggatgcagcaattggcacagttacaacagcatcaaaatcaattgcagcaggcgcatcagcagatgttacaagcacaattacagcagcaagcccgaaactgtggtcaattaaaaacccgaacctgtatacagttagaacagaagttctgaacggaggcaaagttctggatacatatgatacagaatatggctttcgctggacaggctttgatgcaacatcaggcttttcactgaatggcgaaaaagtcaaactgaaaggcgttagcatgcatcatgatcaaggctcacttggcgcagttgcaaatagacgcgcaattgaaagacaagtcgaaatcctgcaaaaaatgggcgtcaatagcattcgcacaacacataatccggcagcaaaagcactgattgatgtctgcaatgaaaaaggcgttctggttgtcgaagaagtctttgatatgtggaaccgcagcaaaaatggcaacacggaagattatggcaaatggtttggccaagcaattgcaggcgataatgcagttctgggaggcgataaagatgaaacatgggcgaaatttgatcttacatcaacaattaaccgcgatagaaatgcaccgtcagttattatgtggtcactgggcaatgaaatgatggaaggcatttcaggctcagtttcaggctttccggcaacatcagcaaaactggttgcatggacaaaagcagcagattcaacaagaccgatgacatatggcgataacaaaattaaagcgaactggaacgaatcaaatacaatgggcgataatctgacagcaaatggcggagttgttggcacaaattattcagatggcgcaaactatgataaaattcgtacaacacatccgtcatgggcaatttatggctcagaaacagcatcagcgattaatagccgtggcatttataatagaacaacaggcggagcacaatcatcagataaacagctgacaagctatgataattcagcagttggctggggagcagttgcatcatcagcatggtatgatgttgttcagagagattttgtcgcaggcacatatgtttggacaggatttgattatctgggcgaaccgacaccgtggaatggcacaggctcaggcgcagttggctcatggccgtcaccgaaaaatagctattttggcatcgttgatacagcaggctttccgaaagatacatattatttttatcagagccagtggaatgatgatgttcatacactgcatattcttccggcatggaatgaaaatgttgttgcaaaaggctcaggcaataatgttccggttgtcgtttatacagatgcagcgaaagtgaaactgtattttacaccgaaaggctcaacagaaaaaagactgatcggcgaaaaatcatttacaaaaaaaacaacagcggcaggctatacatatcaagtctatgaaggcagcgataaagattcaacagcgcataaaaacatgtatctgacatggaatgttccgtgggcagaaggcacaatttcagcggaagcgtatgatgaaaataatcgcctgattccggaaggcagcacagaaggcaacgcatcagttacaacaacaggcaaagcagcaaaactgaaagcagatgcggatcgcaaaacaattacagcggatggcaaagatctgtcatatattgaagtcgatgtcacagatgcaaatggccatattgttccggatgcagcaaatagagtcacatttgatgttaaaggcgcaggcaaactggttggcgttgataatggctcatcaccggatcatgattcatatcaagcggataaccgcaaagcattttcaggcaaagtcctggcaattgttcagtcaacaaaagaagcaggcgaaattacagttacagcaaaagcagatggcctgcaatcaagcacagttaaaattgcaacaacagcagttccgggaacaagcacagaaaaaacagtccgcagcttttattacagccgcaactattatgtcaaaacaggcaacaaaccgattctgccgtcagatgttgaagttcgctattcagatggaacaagcgatagacaaaacgttacatgggatgcagtttcagatgatcaaattgcaaaagcaggctcattttcagttgcaggcacagttgcaggccaaaaaattagcgttcgcgtcacaatgattgatgaaattggcgcactg

SEQ ID NO: 11 - DNA, 3114 bp, Bifidobacterium bifidum
  source 1..3114: mol_type = other DNA
gttgaagatgcaacaagaagcgatagcacaacacaaatgtcatcaacaccggaagttgtttattcatcagcggtcgatagcaaacaaaatcgcacaagcgattttgatgcgaactggaaatttatgctgtcagatagcgttcaagcacaagatccggcatttgatgattcagcatggcaacaagttgatctgccgcatgattatagcatcacacagaaatatagccaaagcaatgaagcagaatcagcatatcttccgggaggcacaggctggtatagaaaaagctttacaattgatagagatctggcaggcaaacgcattgcgattaattttgatggcgtctatatgaatgcaacagtctggtttaatggcgttaaactgggcacacatccgtatggctattcaccgttttcatttgatctgacaggcaatgcaaaatttggcggagaaaacacaattgtcgtcaaagttgaaaatagactgccgtcatcaagatggtattcaggcagcggcatttatagagatgttacactgacagttacagatggcgttcatgttggcaataatggcgtcgcaattaaaacaccgtcactggcaacacaaaatggcggagatgtcacaatgaacctgacaacaaaagtcgcgaatgatacagaagcagcagcgaacattacactgaaacagacagtttttccgaaaggcggaaaaacggatgcagcaattggcacagttacaacagcatcaaaatcaattgcagcaggcgcatcagcagatgttacaagcacaattacagcagcaagcccgaaactgtggtcaattaaaaacccgaacctgtatacagttagaacagaagttctgaacggaggcaaagttctggatacatatgatacagaatatggctttcgctggacaggctttgatgcaacatcaggcttttcactgaatggcgaaaaagtcaaactgaaaggcgttagcatgcatcatgatcaaggctcacttggcgcagttgcaaatagacgcgcaattgaaagacaagtcgaaatcctgcaaaaaatgggcgtcaatagcattcgcacaacacataatccggcagcaaaagcactgattgatgtctgcaatgaaaaaggcgttctggttgtcgaagaagtctttgatatgtggaaccgcagcaaaaatggcaacacggaagattatggcaaatggtttggccaagcaattgcaggcgataatgcagttctgggaggcgataaagatgaaacatgggcgaaatttgatcttacatcaacaattaaccgcgatagaaatgcaccgtcagttattatgtggtcactgggcaatgaaatgatggaaggcatttcaggctcagtttcaggctttccggcaacatcagcaaaactggttgcatggacaaaagcagcagattcaacaagaccgatgacatatggcgataacaaaattaaagcgaactggaacgaatcaaatacaatgggcgataatctgacagcaaatggcggagttgttggcacaaattattcagatggcgcaaactatgataaaattcgtacaacacatccgtcatgggcaatttatggctcagaaacagcatcagcgattaatagccgtggcatttataatagaacaacaggcggagcacaatcatcagataaacagctgacaagctatgataattcagcagttggctggggagcagttgcatcatcagcatggtatgatgttgttcagagagattttgtcgcaggcacatatgtttggacaggatttgattatctgggcgaaccgacaccgtggaatggcacaggctcaggcgcagttggctcatggccgtcaccgaaaaatagctattttggcatcgttgatacagcaggctttccgaaagatacatattatttttatcagagccagtggaatgatgatgttcatacactgcatattcttccggcatggaatgaaaatgttgttgcaaaaggctcaggcaataatgttccggttgtcgtttatacagatgcagcgaaagtgaaactgtattttacaccgaaaggctcaacagaaaaaagactgatcggcgaaaaatcatttacaaaaaaaacaacagcggcaggctatacatatcaagtctatgaaggcagcgataaagattcaacagcgcataaaaacatgtatctgacatggaatgttccgtgggcagaaggcacaatttcagcggaagcgtatgatgaaaataatcgcctgattccggaaggcagcacagaaggcaacgcatcagttacaacaacaggcaaagcagcaaaactgaaagcagatgcggatcgcaaaacaattacagcggatggcaaagatctgtcatatattgaagtcgatgtcacagatgcaaatggccatattgttccggatgcagcaaatagagtcacatttgatgttaaaggcgcaggcaaactggttggcgttgataatggctcatcaccggatcatgattcatatcaagcggataaccgcaaagcattttcaggcaaagtcctggcaattgttcagtcaacaaaagaagcaggcgaaattacagttacagcaaaagcagatggcctgcaatcaagcacagttaaaattgcaacaacagcagttccgggaacaagcacagaaaaaacagtccgcagcttttattacagccgcaactattatgtcaaaacaggcaacaaaccgattctgccgtcagatgttgaagttcgctattcagatggaacaagcgatagacaaaacgttacatgggatgcagtttcagatgatcaaattgcaaaagcaggctcattttcagttgcaggcacagttgcaggccaaaaaattagcgttcgcgtcacaatgattgatgaaattggcgcactgctgaattattcagcaagcacaccggttggcacaccggcagttcttccgggatcaagaccggcagtcctgccggatggcacagtcacatcagcaaattttgcagtccattggacaaaaccggcagatacagtctataatacagcaggcacagtcaaagtaccgggaacagcaacagtttttggcaaagaatttaaagtcacagcgacaattagagttcaa

SEQ ID NO: 12 - DNA, 3426 bp, Bifidobacterium bifidum
  source 1..3426: mol_type = other DNA
gttgaagatgcaacaagaagcgatagcacaacacaaatgtcatcaacaccggaagttgtttattcatcagcggtcgatagcaaacaaaatcgcacaagcgattttgatgcgaactggaaatttatgctgtcagatagcgttcaagcacaagatccggcatttgatgattcagcatggcaacaagttgatctgccgcatgattatagcatcacacagaaatatagccaaagcaatgaagcagaatcagcatatcttccgggaggcacaggctggtatagaaaaagctttacaattgatagagatctggcaggcaaacgcattgcgattaattttgatggcgtctatatgaatgcaacagtctggtttaatggcgttaaactgggcacacatccgtatggctattcaccgttttcatttgatctgacaggcaatgcaaaatttggcggagaaaacacaattgtcgtcaaagttgaaaatagactgccgtcatcaagatggtattcaggcagcggcatttatagagatgttacactgacagttacagatggcgttcatgttggcaataatggcgtcgcaattaaaacaccgtcactggcaacacaaaatggcggagatgtcacaatgaacctgacaacaaaagtcgcgaatgatacagaagcagcagcgaacattacactgaaacagacagtttttccgaaaggcggaaaaacggatgcagcaattggcacagttacaacagcatcaaaatcaattgcagcaggcgcatcagcagatgttacaagcacaattacagcagcaagcccgaaactgtggtcaattaaaaacccgaacctgtatacagttagaacagaagttctgaacggaggcaaagttctggatacatatgatacagaatatggctttcgctggacaggctttgatgcaacatcaggcttttcactgaatggcgaaaaagtcaaactgaaaggcgttagcatgcatcatgatcaaggctcacttggcgcagttgcaaatagacgcgcaattgaaagacaagtcgaaatcctgcaaaaaatgggcgtcaatagcattcgcacaacacataatccggcagcaaaagcactgattgatgtctgcaatgaaaaaggcgttctggttgtcgaagaagtctttgatatgtggaaccgcagcaaaaatggcaacacggaagattatggcaaatggtttggccaagcaattgcaggcgataatgcagttctgggaggcgataaagatgaaacatgggcgaaatttgatcttacatcaacaattaaccgcgatagaaatgcaccgtcagttattatgtggtcactgggcaatgaaatgatggaaggcatttcaggctcagtttcaggctttccggcaacatcagcaaaactggttgcatggacaaaagcagcagattcaacaagaccgatgacatatggcgataacaaaattaaagcgaactggaacgaatcaaatacaatgggcgataatctgacagcaaatggcggagttgttggcacaaattattcagatggcgcaaactatgataaaattcgtacaacacatccgtcatgggcaatttatggctcagaaacagcatcagcgattaatagccgtggcatttataatagaacaacaggcggagcacaatcatcagataaacagctgacaagctatgataattcagcagttggctggggagcagttgcatcatcagcatggtatgatgttgttcagagagattttgtcgcaggcacatatgtttggacaggatttgattatctgggcgaaccgacaccgtggaatggcacaggctcaggcgcagttggctcatggccgtcaccgaaaaatagctattttggcatcgttgatacagcaggctttccgaaagatacatattatttttatcagagccagtggaatgatgatgttcatacactgcatattcttccggcatggaatgaaaatgttgttgcaaaaggctcaggcaataatgttccggttgtcgtttatacagatgcagcgaaagtgaaactgtattttacaccgaaaggctcaacagaaaaaagactgatcggcgaaaaatcatttacaaaaaaaacaacagcggcaggctatacatatcaagtctatgaaggcagcgataaagattcaacagcgcataaaaacatgtatctgacatggaatgttccgtgggcagaaggcacaatttcagcggaagcgtatgatgaaaataatcgcctgattccggaaggcagcacagaaggcaacgcatcagttacaacaacaggcaaagcagcaaaactgaaagcagatgcggatcgcaaaacaattacagcggatggcaaagatctgtcatatattgaagtcgatgtcacagatgcaaatggccatattgttccggatgcagcaaatagagtcacatttgatgttaaaggcgcaggcaaactggttggcgttgataatggctcatcaccggatcatgattcatatcaagcggataaccgcaaagcattttcaggcaaagtcctggcaattgttcagtcaacaaaagaagcaggcgaaattacagttacagcaaaagcagatggcctgcaatcaagcacagttaaaattgcaacaacagcagttccgggaacaagcacagaaaaaacagtccgcagcttttattacagccgcaactattatgtcaaaacaggcaacaaaccgattctgccgtcagatgttgaagttcgctattcagatggaacaagcgatagacaaaacgttacatgggatgcagtttcagatgatcaaattgcaaaagcaggctcattttcagttgcaggcacagttgcaggccaaaaaattagcgttcgcgtcacaatgattgatgaaattggcgcactgctgaattattcagcaagcacaccggttggcacaccggcagttcttccgggatcaagaccggcagtcctgccggatggcacagtcacatcagcaaattttgcagtccattggacaaaaccggcagatacagtctataatacagcaggcacagtcaaagtaccgggaacagcaacagtttttggcaaagaatttaaagtcacagcgacaattagagttcaaagaagccaagttacaattggctcatcagtttcaggaaatgcactgagactgacacaaaatattccggcagataaacaatcagatacactggatgcgattaaagatggctcaacaacagttgatgcaaatacaggcggaggcgcaaatccgtcagcatggacaaattgggcatattcaaaagcaggccataacacagcggaaattacatttgaatatgcgacagaacaacaactgggccagatcgtcatgtatttttttcgcgatagcaatgcagttagatttccggatgctggcaaaacaaaaattcagatc

SEQ ID NO: 13 - DNA, 3633 bp, Bifidobacterium bifidum
  source 1..3633: mol_type = other DNA
gttgaagatgcaacaagaagcgatagcacaacacaaatgtcatcaacaccggaagttgtttattcatcagcggtcgatagcaaacaaaatcgcacaagcgattttgatgcgaactggaaatttatgctgtcagatagcgttcaagcacaagatccggcatttgatgattcagcatggcaacaagttgatctgccgcatgattatagcatcacacagaaatatagccaaagcaatgaagcagaatcagcatatcttccgggaggcacaggctggtatagaaaaagctttacaattgatagagatctggcaggcaaacgcattgcgattaattttgatggcgtctatatgaatgcaacagtctggtttaatggcgttaaactgggcacacatccgtatggctattcaccgttttcatttgatctgacaggcaatgcaaaatttggcggagaaaacacaattgtcgtcaaagttgaaaatagactgccgtcatcaagatggtattcaggcagcggcatttatagagatgttacactgacagttacagatggcgttcatgttggcaataatggcgtcgcaattaaaacaccgtcactggcaacacaaaatggcggagatgtcacaatgaacctgacaacaaaagtcgcgaatgatacagaagcagcagcgaacattacactgaaacagacagtttttccgaaaggcggaaaaacggatgcagcaattggcacagttacaacagcatcaaaatcaattgcagcaggcgcatcagcagatgttacaagcacaattacagcagcaagcccgaaactgtggtcaattaaaaacccgaacctgtatacagttagaacagaagttctgaacggaggcaaagttctggatacatatgatacagaatatggctttcgctggacaggctttgatgcaacatcaggcttttcactgaatggcgaaaaagtcaaactgaaaggcgttagcatgcatcatgatcaaggctcacttggcgcagttgcaaatagacgcgcaattgaaagacaagtcgaaatcctgcaaaaaatgggcgtcaatagcattcgcacaacacataatccggcagcaaaagcactgattgatgtctgcaatgaaaaaggcgttctggttgtcgaagaagtctttgatatgtggaaccgcagcaaaaatggcaacacggaagattatggcaaatggtttggccaagcaattgcaggcgataatgcagttctgggaggcgataaagatgaaacatgggcgaaatttgatcttacatcaacaattaaccgcgatagaaatgcaccgtcagttattatgtggtcactgggcaatgaaatgatggaaggcatttcaggctcagtttcaggctttccggcaacatcagcaaaactggttgcatggacaaaagcagcagattcaacaagaccgatgacatatggcgataacaaaattaaagcgaactggaacgaatcaaatacaatgggcgataatctgacagcaaatggcggagttgttggcacaaattattcagatggcgcaaactatgataaaattcgtacaacacatccgtcatgggcaatttatggctcagaaacagcatcagcgattaatagccgtggcatttataatagaacaacaggcggagcacaatcatcagataaacagctgacaagctatgataattcagcagttggctggggagcagttgcatcatcagcatggtatgatgttgttcagagagattttgtcgcaggcacatatgtttggacaggatttgattatctgggcgaaccgacaccgtggaatggcacaggctcaggcgcagttggctcatggccgtcaccgaaaaatagctattttggcatcgttgatacagcaggctttccgaaagatacatattatttttatcagagccagtggaatgatgatgttcatacactgcatattcttccggcatggaatgaaaatgttgttgcaaaaggctcaggcaataatgttccggttgtcgtttatacagatgcagcgaaagtgaaactgtattttacaccgaaaggctcaacagaaaaaagactgatcggcgaaaaatcatttacaaaaaaaacaacagcggcaggctatacatatcaagtctatgaaggcagcgataaagattcaacagcgcataaaaacatgtatctgacatggaatgttccgtgggcagaaggcacaatttcagcggaagcgtatgatgaaaataatcgcctgattccggaaggcagcacagaaggcaacgcatcagttacaacaacaggcaaagcagcaaaactgaaagcagatgcggatcgcaaaacaattacagcggatggcaaagatctgtcatatattgaagtcgatgtcacagatgcaaatggccatattgttccggatgcagcaaatagagtcacatttgatgttaaaggcgcaggcaaactggttggcgttgataatggctcatcaccggatcatgattcatatcaagcggataaccgcaaagcattttcaggcaaagtcctggcaattgttcagtcaacaaaagaagcaggcgaaattacagttacagcaaaagcagatggcctgcaatcaagcacagttaaaattgcaacaacagcagttccgggaacaagcacagaaaaaacagtccgcagcttttattacagccgcaactattatgtcaaaacaggcaacaaaccgattctgccgtcagatgttgaagttcgctattcagatggaacaagcgatagacaaaacgttacatgggatgcagtttcagatgatcaaattgcaaaagcaggctcattttcagttgcaggcacagttgcaggccaaaaaattagcgttcgcgtcacaatgattgatgaaattggcgcactgctgaattattcagcaagcacaccggttggcacaccggcagttcttccgggatcaagaccggcagtcctgccggatggcacagtcacatcagcaaattttgcagtccattggacaaaaccggcagatacagtctataatacagcaggcacagtcaaagtaccgggaacagcaacagtttttggcaaagaatttaaagtcacagcgacaattagagttcaaagaagccaagttacaattggctcatcagtttcaggaaatgcactgagactgacacaaaatattccggcagataaacaatcagatacactggatgcgattaaagatggctcaacaacagttgatgcaaatacaggcggaggcgcaaatccgtcagcatggacaaattgggcatattcaaaagcaggccataacacagcggaaattacatttgaatatgcgacagaacaacaactgggccagatcgtcatgtatttttttcgcgatagcaatgcagttagatttccggatgctggcaaaacaaaaattcagatcagcgcagatggcaaaaattggacagatctggcagcaacagaaacaattgcagcgcaagaatcaagcgatagagtcaaaccgtatacatatgattttgcaccggttggcgcaacatttgttaaagtgacagtcacaaacgcagatacaacaacaccgtcaggcgttgtttgcgcaggcctgacagaaattgaactgaaaacagcgaca

SEQ ID NO: 14 - DNA, 3888 bp, Bifidobacterium bifidum
  source 1..3888: mol_type = other DNA
gttgaagatgcaacaagaagcgatagcacaacacaaatgtcatcaacaccggaagttgtttattcatcagcggtcgatagcaaacaaaatcgcacaagcgattttgatgcgaactggaaatttatgctgtcagatagcgttcaagcacaagatccggcatttgatgattcagcatggcaacaagttgatctgccgcatgattatagcatcacacagaaatatagccaaagcaatgaagcagaatcagcatatcttccgggaggcacaggctggtatagaaaaagctttacaattgatagagatctggcaggcaaacgcattgcgattaattttgatggcgtctatatgaatgcaacagtctggtttaatggcgttaaactgggcacacatccgtatggctattcaccgttttcatttgatctgacaggcaatgcaaaatttggcggagaaaacacaattgtcgtcaaagttgaaaatagactgccgtcatcaagatggtattcaggcagcggcatttatagagatgttacactgacagttacagatggcgttcatgttggcaataatggcgtcgcaattaaaacaccgtcactggcaacacaaaatggcggagatgtcacaatgaacctgacaacaaaagtcgcgaatgatacagaagcagcagcgaacattacactgaaacagacagtttttccgaaaggcggaaaaacggatgcagcaattggcacagttacaacagcatcaaaatcaattgcagcaggcgcatcagcagatgttacaagcacaattacagcagcaagcccgaaactgtggtcaattaaaaacccgaacctgtatacagttagaacagaagttctgaacggaggcaaagttctggatacatatgatacagaatatggctttcgctggacaggctttgatgcaacatcaggcttttcactgaatggcgaaaaagtcaaactgaaaggcgttagcatgcatcatgatcaaggctcacttggcgcagttgcaaatagacgcgcaattgaaagacaagtcgaaatcctgcaaaaaatgggcgtcaatagcattcgcacaacacataatccggcagcaaaagcactgattgatgtctgcaatgaaaaaggcgttctggttgtcgaagaagtctttgatatgtggaaccgcagcaaaaatggcaacacggaagattatggcaaatggtttggccaagcaattgcaggcgataatgcagttctgggaggcgataaagatgaaacatgggcgaaatttgatcttacatcaacaattaaccgcgatagaaatgcaccgtcagttattatgtggtcactgggcaatgaaatgatggaaggcatttcaggctcagtttcaggctttccggcaacatcagcaaaactggttgcatggacaaaagcagcagattcaacaagaccgatgacatatggcgataacaaaattaaagcgaactggaacgaatcaaatacaatgggcgataatctgacagcaaatggcggagttgttggcacaaattattcagatggcgcaaactatgataaaattcgtacaacacatccgtcatgggcaatttatggctcagaaacagcatcagcgattaatagccgtggcatttataatagaacaacaggcggagcacaatcatcagataaacagctgacaagctatgataattcagcagttggctggggagcagttgcatcatcagcatggtatgatgttgttcagagagattttgtcgcaggcacatatgtttggacaggatttgattatctgggcgaaccgacaccgtggaatggcacaggctcaggcgcagttggctcatggccgtcaccgaaaaatagctattttggcatcgttgatacagcaggctttccgaaagatacatattatttttatcagagccagtggaatgatgatgttcatacactgcatattcttccggcatggaatgaaaatgttgttgcaaaaggctcaggcaataatgttccggttgtcgtttatacagatgcagcgaaagtgaaactgtattttacaccgaaaggctcaacagaaaaaagactgatcggcgaaaaatcatttacaaaaaaaacaacagcggcaggctatacatatcaagtctatgaaggcagcgataaagattcaacagcgcataaaaacatgtatctgacatggaatgttccgtgggcagaaggcacaatttcagcggaagcgtatgatgaaaataatcgcctgattccggaaggcagcacagaaggcaacgcatcagttacaacaacaggcaaagcagcaaaactgaaagcagatgcggatcgcaaaacaattacagcggatggcaaagatctgtcatatattgaagtcgatgtcacagatgcaaatggccatattgttccggatgcagcaaatagagtcacatttgatgttaaaggcgcaggcaaactggttggcgttgataatggctcatcaccggatcatgattcatatcaagcggataaccgcaaagcattttcaggcaaagtcctggcaattgttcagtcaacaaaagaagcaggcgaaattacagttacagcaaaagcagatggcctgcaatcaagcacagttaaaattgcaacaacagcagttccgggaacaagcacagaaaaaacagtccgcagcttttattacagccgcaactattatgtcaaaacaggcaacaaaccgattctgccgtcagatgttgaagttcgctattcagatggaacaagcgatagacaaaacgttacatgggatgcagtttcagatgatcaaattgcaaaagcaggctcattttcagttgcaggcacagttgcaggccaaaaaattagcgttcgcgtcacaatgattgatgaaattggcgcactgctgaattattcagcaagcacaccggttggcacaccggcagttcttccgggatcaagaccggcagtcctgccggatggcacagtcacatcagcaaattttgcagtccattggacaaaaccggcagatacagtctataatacagcaggcacagtcaaagtaccgggaacagcaacagtttttggcaaagaatttaaagtcacagcgacaattagagttcaaagaagccaagttacaattggctcatcagtttcaggaaatgcactgagactgacacaaaatattccggcagataaacaatcagatacactggatgcgattaaagatggctcaacaacagttgatgcaaatacaggcggaggcgcaaatccgtcagcatggacaaattgggcatattcaaaagcaggccataacacagcggaaattacatttgaatatgcgacagaacaacaactgggccagatcgtcatgtatttttttcgcgatagcaatgcagttagatttccggatgctggcaaaacaaaaattcagatcagcgcagatggcaaaaattggacagatctggcagcaacagaaacaattgcagcgcaagaatcaagcgatagagtcaaaccgtatacatatgattttgcaccggttggcgcaacatttgttaaagtgacagtcacaaacgcagatacaacaacaccgtcaggcgttgtttgcgcaggcctgacagaaattgaactgaaaacagcgacaagcaaatttgtcacaaatacatcagcagcactgtcatcacttacagtcaatggcacaaaagtttcagattcagttctggcagcaggctcatataacacaccggcaattatcgcagatgttaaagcggaaggcgaaggcaatgcaagcgttacagtccttccggcacatgataatgttattcgcgtcattacagaaagcgaagatcatgtcacacgcaaaacatttacaatcaacctgggcacagaacaagaattt

SEQ ID NO: 15 - DNA, 30 bp, synthetic construct
  source 1..30: mol_type = other DNA; note = Synthetic DNA primer
ggggtaactagtggaagatgcaacaagaag

SEQ ID NO: 16 - DNA, 35 bp, synthetic construct
  source 1..35: mol_type = other DNA; note = Synthetic DNA primer
gcgcttaattaattatgttttttctgtgcttgttc

SEQ ID NO: 17 - DNA, 38 bp, synthetic construct
  source 1..38: mol_type = other DNA; note = Synthetic PCR primer
gcgcttaattaattacagtgcgccaatttcatcaatca

SEQ ID NO: 18 - DNA, 35 bp, synthetic construct
  source 1..35: mol_type = other DNA; note = Synthetic PCR primer
gcgcttaattaattattgaactctaattgtcgctg

SEQ ID NO: 19 - DNA, 36 bp, synthetic construct
  source 1..36: mol_type = other DNA; note = Synthetic PCR primer
gcgcttaattaattatgtcgctgttttcagttcaat

SEQ ID NO: 20 - DNA, 35 bp, synthetic construct
  source 1..35: mol_type = other DNA; note = Synthetic PCR primer
gcgcttaattaattaaaattcttgttctgtgccca

SEQ ID NO: 21 - DNA, 38 bp, synthetic construct
  source 1..38: mol_type = other DNA; note = Synthetic PCR primer
gcgcttaattaattatctcagtctaatttcgcttgcgc

SEQ ID NO: 22 - protein, 1720 aa, Bifidobacterium bifidum
VEDATRSDSTTQMSSTPEVVYSSAVDSKQNRTSDFDANWKFMLSDSVQAQDPAFDDSAWQQVDLPHDYSITQKYSQSNEAESAYLPGGTGWYRKSFTIDRDLAGKRIAINFDGVYMNATVWFNGVKLGTHPYGYSPFSFDLTGNAKFGGENTIVVKVENRLPSSRWYSGSGIYRDVTLTVTDGVHVGNNGVAIKTPSLATQNGGDVTMNLTTKVANDTEAAANITLKQTVFPKGGKTDAAIGTVTTASKSIAAGASADVTSTITAASPKLWSIKNPNLYTVRTEVLNGGKVLDTYDTEYGFRWTGFDATSGFSLNGEKVKLKGVSMHHDQGSLGAVANRRAIERQVEILQKMGVNSIRTTHNPAAKALIDVCNEKGVLVVEEVFDMWNRSKNGNTEDYGKWFGQAIAGDNAVLGGDKDETWAKFDLTSTINRDRNAPSVIMWSLGNEMMEGISGSVSGFPATSAKLVAWTKAADSTRPMTYGDNKIKANWNESNTMGDNLTANGGVVGTNYSDGANYDKIRTTHPSWAIYGSETASAINSRGIYNRTTGGAQSSDKQLTSYDNSAVGWGAVASSAWYDVVQRDFVAGTYVWTGFDYLGEPTPWNGTGSGAVGSWPSPKNSYFGIVDTAGFPKDTYYFYQSQWNDDVHTLHILPAWNENVVAKGSGNNVPVVVYTDAAKVKLYFTPKGSTEKRLIGEKSFTKKTTAAGYTYQVYEGSDKDSTAHKNMYLTWNVPWAEGTISAEAYDENNRLIPEGSTEGNASVTTTGKAAKLKADADRKTITADGKDLSYIEVDVTDANGHIVPDAANRVTFDVKGAGKLVGVDNGSSPDHDSYQADNRKAFSGKVLAIVQSTKEAGEITVTAKADGLQSSTVKIATTAVPGTSTEKTVRSFYYSRNYYVKTGNKPILPSDVEVRYSDGTSDRQNVTWDAVSDDQIAKAGSFSVAGTVAGQKISVRVTMIDEIGALLNYSASTPVGTPAVLPGSRPAVLPDGTVTSANFAVHWTKPADTVYNTAGTVKVPGTATVFGKEFKVTATIRVQRSQVTIGSSVSGNALRLTQNIPADKQSDTLDAIKDGSTTVDANTGGGANPSAWTNWAYSKAGHNTAEITFEYATEQQLGQIVMYFFRDSNAVRFPDAGKTKIQISADGKNWTDLAATETIAAQESSDRVKPYTYDFAPVGATFVKVTVTNADTTTPSGVVCAGLTEIELKTATSKFVTNTSAALSSLTVNGTKVSDSVLAAGSYNTPAIIADVKAEGEGNASVTVLPAHDNVIRVITESEDHVTRKTFTINLGTEQEFPADSDERDYPAADMTVTVGSEQTSGTATEGPKKFAVDGNTSTYWHSNWTPTTVNDLWIAFELQKPTKLDALRYLPRPAGSKNGSVTEYKVQVSDDGTNWTDAGSGTWTTDYGWKLAEFNQPVTTKHVRLKAVHTYADSGNDKFMSASEIRLRKAVDTTDISGATVTVPAKLTVDRVDADHPATFATKDVTVTLGDATLRYGVDYLLDYAGNTAVGKATVTVRGIDKYSGTVAKTFTIELKNAPAPEPTLTSVSVKTKPSKLTYVVGDAFDPAGLVLQHDRQADRPPQPLVGEQADERGLTCGTRCDRVEQLRKHENREAHRTGLDHLEFVGAADGAVGEQATFKVHVHADQGDGRHDDADERDIDPHVPVDHAVGELARAACHHVIGLRVDTHRLKASGFQIPADDMAEIDRITGFHRFERHVG

SEQ ID NO: 23 - protein, 30 aa, Bifidobacterium bifidum
  source 1..30: note = Signal sequence of extracellular lactase from Bifidobacterium bifidum DSM20215
VRSKKLWISLLFALALIFTMAFGSTSSAQA